European Patent Application EP 4 183 415 A1, published May 24, 2023. Title: TRPV4 antagonist for use in the treatment of ophthalmic disease. Applicant: RaQualia Pharma Inc. The sequence listing filed with the application follows.

SEQUENCE LISTING (8 sequences)

SEQ ID NO: 1 - DNA, 3228 bp, Homo sapiens
attcaggaagcgcggatctcccggccgccggcgcccagccgtcccggaggctgagcagtgcagacgggcctggggcaggcatggcggattccagcgaaggcccccgcgcggggcccggggaggtggctgagctccccggggatgagagtggcaccccaggtggggaggcttttcctctctcctccctggccaatctgtttgagggggaggatggctccctttcgccctcaccggctgatgccagtcgccctgctggcccaggcgatgggcgaccaaatctgcgcatgaagttccagggcgccttccgcaagggggtgcccaaccccatcgatctgctggagtccaccctatatgagtcctcggtggtgcctgggcccaagaaagcacccatggactcactgtttgactacggcacctatcgtcaccactccagtgacaacaagaggtggaggaagaagatcatagagaagcagccgcagagccccaaagcccctgcccctcagccgccccccatcctcaaagtcttcaaccggcctatcctctttgacatcgtgtcccggggctccactgctgacctggacgggctgctcccattcttgctgacccacaagaaacgcctaactgatgaggagtttcgagagccatctacggggaagacctgcctgcccaaggccttgctgaacctgagcaatggccgcaacgacaccatccctgtgctgctggacatcgcggagcgcaccggcaacatgagggagttcattaactcgcccttccgtgacatctactatcgaggtcagacagccctgcacatcgccattgagcgtcgctgcaaacactacgtggaacttctcgtggcccagggagctgatgtccacgcccaggcccgtgggcgcttcttccagcccaaggatgaggggggctacttctactttggggagctgcccctgtcgctggctgcctgcaccaaccagccccacattgtcaactacctgacggagaacccccacaagaaggcggacatgcggcgccaggactcgcgaggcaacacagtgctgcatgcgctggtggccattgctgacaacacccgtgagaacaccaagtttgttaccaagatgtacgacctgctgctgctcaagtgtgcccgcctcttccccgacagcaacctggaggccgtgctcaacaacgacggcctctcgcccctcatgatggctgccaagacgggcaagattgggatctttcagcacatcatccggcgggaggtgacggatgaggacacacggcacctgtcccgcaagttcaaggactgggcctatgggccagtgtattcctcgctttatgacctctcctccctggacacgtgtggggaagaggcctccgtgctggagatcctggtgtacaacagcaagattgagaaccgccacgagatgctggctgtggagcccatcaatgaactgctgcgggacaagtggcgcaagttcggggccgtctccttctacatcaacgtggtctcctacctgtgtgccatggtcatcttcactctcaccgcctactaccagccgctggagggcacaccgccgtacccttaccgcaccacggtggactacctgcggctggctggcgaggtcattacgctcttcactggggtcctgttcttcttcaccaacatcaaagacttgttcatgaagaaatgccctggagtgaattctctcttcattgatggctccttccagctgctctacttcatctactctgtcctggtgatcgtctcagcagccctctacctggcagggatcgaggcctacctggccgtgatggtctttgccctggtcctgggctggatgaatgccctttacttcacccgtgggctgaagctgacggggacctatagcatcatgatccagaagattctcttcaaggaccttttccgattcctgctcgtctacttgctcttcatgatcggctacgcttcagccctggtctccctcctgaacccgtgtgccaacatgaaggtgtgcaatgaggaccagaccaactgcacagtgcccacttacccctcgtgccgtgacagcgagaccttcagcaccttcctcctggacctgtttaagctgaccatcggcatgggcgacctggagatgctgagcagcaccaagtaccccgtggtcttcatcatcctgctggtgacctacatcatcctcacctttgtgctgctcctcaacatgctcattgccctcatgggcgagacagtgggccaggtctccaaggagagcaagcacatctggaagctgcagtgggccaccaccatcctggacattgagcgctccttccccgtattcctgaggaaggccttccgctctggggagatggtcaccgtgggcaagagctcggacggcactcctgaccgcaggtggtgcttcagggtggatgaggtgaactggtctcactggaaccagaacttgggcatcatcaacgaggacccgggcaagaatgagacctaccagtattatggcttctcgcataccgtgggccgcctccgcagggatcgctggtcctcggtggtaccccgcgtggtggaactgaacaagaactcgaacccggacgaggtggtggtgcctctggacagcatggggaacccccgctgcgatggccaccagcagggttacccccgcaagtggaggactgatgacgccccgctctagggactgcagcccagccccagcttctctgcccactcatttctagtccagccgcatttcagcagtgccttctggggtgtccccccacaccctgctttggccccagaggcgagggaccagtggaggtgccagggaggccccaggaccctgtggtcccctggctctgcctccccaccctggggtgggggctcccggccacctgtcttgctcctatggagtcacataagccaacgccagagcccctccacctcaggccccagcccctgcctctccattatttatttgctctgctctcaggaagcgacgtgacccctgccccagctggaacctggcagaggccttaggaccccgttccaagtgcactgcccggccaagccccagcctcagcctgcgcctgagctgcatgcgccaccatttttggcagcgtggcagctttgcaaggggctggggccctcggcgtggggccatgccttctgtgtgttctgtagtgtctgggatttgccggtgctcaataaatgtttattcattgacggtg

SEQ ID NO: 2 - DNA, 3012 bp, Homo sapiens
gctgagcagtgcagacgggcctggggcaggcatggcggattccagcgaaggcccccgcgcggggcccggggaggtggctgagctccccggggatgagagtggcaccccaggtggggaggcttttcctctctcctccctggccaatctgtttgagggggaggatggctccctttcgccctcaccggctgatgccagtcgccctgctggcccaggcgatgggcgaccaaatctgcgcatgaagttccagggcgccttccgcaagggggtgcccaaccccatcgatctgctggagtccaccctatatgagtcctcggtggtgcctgggcccaagaaagcacccatggactcactgtttgactacggcacctatcgtcaccactccagtgacaacaagaggtggaggaagaagatcatagagaagcagccgcagagccccaaagcccctgcccctcagccgccccccatcctcaaagtcttcaaccggcctatcctctttgacatcgtgtcccggggctccactgctgacctggacgggctgctcccattcttgctgacccacaagaaacgcctaactgatgaggagtttcgagagccatctacggggaagacctgcctgcccaaggccttgctgaacctgagcaatggccgcaacgacaccatccctgtgctgctggacatcgcggagcgcaccggcaacatgagggagttcattaactcgcccttccgtgacatctactatcgaggtcagacagccctgcacatcgccattgagcgtcgctgcaaacactacgtggaacttctcgtggcccagggagctgatgtccacgcccaggcccgtgggcgcttcttccagcccaaggatgaggggggctacttctactttggggagctgcccctgtcgctggctgcctgcaccaaccagccccacattgtcaactacctgacggagaacccccacaagaaggcggacatgcggcgccaggactcgcgaggcaacacagtgctgcatgcgctggtggccattgctgacaacacccgtgagaacaccaagtttgttaccaagatgtacgacctgctgctgctcaagtgtgcccgcctcttccccgacagcaacctggaggccgtgctcaacaacgacggcctctcgcccctcatgatggctgccaagacgggcaagattgggaaccgccacgagatgctggctgtggagcccatcaatgaactgctgcgggacaagtggcgcaagttcggggccgtctccttctacatcaacgtggtctcctacctgtgtgccatggtcatcttcactctcaccgcctactaccagccgctggagggcacaccgccgtacccttaccgcaccacggtggactacctgcggctggctggcgaggtcattacgctcttcactggggtcctgttcttcttcaccaacatcaaagacttgttcatgaagaaatgccctggagtgaattctctcttcattgatggctccttccagctgctctacttcatctactctgtcctggtgatcgtctcagcagccctctacctggcagggatcgaggcctacctggccgtgatggtctttgccctggtcctgggctggatgaatgccctttacttcacccgtgggctgaagctgacggggacctatagcatcatgatccagaagattctcttcaaggaccttttccgattcctgctcgtctacttgctcttcatgatcggctacgcttcagccctggtctccctcctgaacccgtgtgccaacatgaaggtgtgcaatgaggaccagaccaactgcacagtgcccacttacccctcgtgccgtgacagcgagaccttcagcaccttcctcctggacctgtttaagctgaccatcggcatgggcgacctggagatgctgagcagcaccaagtaccccgtggtcttcatcatcctgctggtgacctacatcatcctcacctttgtgctgctcctcaacatgctcattgccctcatgggcgagacagtgggccaggtctccaaggagagcaagcacatctggaagctgcagtgggccaccaccatcctggacattgagcgctccttccccgtattcctgaggaaggccttccgctctggggagatggtcaccgtgggcaagagctcggacggcactcctgaccgcaggtggtgcttcagggtggatgaggtgaactggtctcactggaaccagaacttgggcatcatcaacgaggacccgggcaagaatgagacctaccagtattatggcttctcgcataccgtgggccgcctccgcagggatcgctggtcctcggtggtaccccgcgtggtggaactgaacaagaactcgaacccggacgaggtggtggtgcctctggacagcatggggaacccccgctgcgatggccaccagcagggttacccccgcaagtggaggactgatgacgccccgctctagggactgcagcccagccccagcttctctgcccactcatttctagtccagccgcatttcagcagtgccttctggggtgtccccccacaccctgctttggccccagaggcgagggaccagtggaggtgccagggaggccccaggaccctgtggtcccctggctctgcctccccaccctggggtgggggctcccggccacctgtcttgctcctatggagtcacataagccaacgccagagcccctccacctcaggccccagcccctgcctctccattatttatttgctctgctctcaggaagcgacgtgacccctgccccagctggaacctggcagaggccttaggaccccgttccaagtgcactgcccggccaagccccagcctcagcctgcgcctgagctgcatgcgccaccatttttggcagcgtggcagctttgcaaggggctggggccctcggcgtggggccatgccttctgtgtgttctgtagtgtctgggatttgccggtgctcaataaatgtttattcattgacggtggaaaaaaaaaaaa

SEQ ID NO: 3 - DNA, 2871 bp, Homo sapiens
gctgagcagtgcagacgggcctggggcaggcatggcggattccagcgaaggcccccgcgcggggcccggggaggtggctgagctccccggggatgagagtggcaccccaggtggggaggcttttcctctctcctccctggccaatctgtttgagggggaggatggctccctttcgccctcaccggctgatgccagtcgccctgctggcccaggcgatgggcgaccaaatctgcgcatgaagttccagggcgccttccgcaagggggtgcccaaccccatcgatctgctggagtccaccctatatgagtcctcggtggtgcctgggcccaagaaagcacccatggactcactgtttgactacggcacctatcgtcaccactccagtgacaacaagaggtggaggaagaagatcatagagaagcagccgcagagccccaaagcccctgcccctcagccgccccccatcctcaaagtcttcaaccggcctatcctctttgacatcgtgtcccggggctccactgctgacctggacgggctgctcccattcttgctgacccacaagaaacgcctaactgatgaggagtttcgagagccatctacggggaagacctgcctgcccaaggccttgctgaacctgagcaatggccgcaacgacaccatccctgtgctgctggacatcgcggagcgcaccggcaacatgagggagttcattaactcgcccttccgtgacatctactatcgaggggagctgcccctgtcgctggctgcctgcaccaaccagccccacattgtcaactacctgacggagaacccccacaagaaggcggacatgcggcgccaggactcgcgaggcaacacagtgctgcatgcgctggtggccattgctgacaacacccgtgagaacaccaagtttgttaccaagatgtacgacctgctgctgctcaagtgtgcccgcctcttccccgacagcaacctggaggccgtgctcaacaacgacggcctctcgcccctcatgatggctgccaagacgggcaagattgggaaccgccacgagatgctggctgtggagcccatcaatgaactgctgcgggacaagtggcgcaagttcggggccgtctccttctacatcaacgtggtctcctacctgtgtgccatggtcatcttcactctcaccgcctactaccagccgctggagggcacaccgccgtacccttaccgcaccacggtggactacctgcggctggctggcgaggtcattacgctcttcactggggtcctgttcttcttcaccaacatcaaagacttgttcatgaagaaatgccctggagtgaattctctcttcattgatggctccttccagctgctctacttcatctactctgtcctggtgatcgtctcagcagccctctacctggcagggatcgaggcctacctggccgtgatggtctttgccctggtcctgggctggatgaatgccctttacttcacccgtgggctgaagctgacggggacctatagcatcatgatccagaagattctcttcaaggaccttttccgattcctgctcgtctacttgctcttcatgatcggctacgcttcagccctggtctccctcctgaacccgtgtgccaacatgaaggtgtgcaatgaggaccagaccaactgcacagtgcccacttacccctcgtgccgtgacagcgagaccttcagcaccttcctcctggacctgtttaagctgaccatcggcatgggcgacctggagatgctgagcagcaccaagtaccccgtggtcttcatcatcctgctggtgacctacatcatcctcacctttgtgctgctcctcaacatgctcattgccctcatgggcgagacagtgggccaggtctccaaggagagcaagcacatctggaagctgcagtgggccaccaccatcctggacattgagcgctccttccccgtattcctgaggaaggccttccgctctggggagatggtcaccgtgggcaagagctcggacggcactcctgaccgcaggtggtgcttcagggtggatgaggtgaactggtctcactggaaccagaacttgggcatcatcaacgaggacccgggcaagaatgagacctaccagtattatggcttctcgcataccgtgggccgcctccgcagggatcgctggtcctcggtggtaccccgcgtggtggaactgaacaagaactcgaacccggacgaggtggtggtgcctctggacagcatggggaacccccgctgcgatggccaccagcagggttacccccgcaagtggaggactgatgacgccccgctctagggactgcagcccagccccagcttctctgcccactcatttctagtccagccgcatttcagcagtgccttctggggtgtccccccacaccctgctttggccccagaggcgagggaccagtggaggtgccagggaggccccaggaccctgtggtcccctggctctgcctccccaccctggggtgggggctcccggccacctgtcttgctcctatggagtcacataagccaacgccagagcccctccacctcaggccccagcccctgcctctccattatttatttgctctgctctcaggaagcgacgtgacccctgccccagctggaacctggcagaggccttaggaccccgttccaagtgcactgcccggccaagccccagcctcagcctgcgcctgagctgcatgcgccaccatttttggcagcgtggcagctttgcaaggggctggggccctcggcgtggggccatgccttctgtgtgttctgtagtgtctgggatttgccggtgctcaataaatgtttattcattgacggtggaaaaaaaaaaaa

SEQ ID NO: 4 - DNA, 3059 bp, Homo sapiens
atggcggattccagcgaaggcccccgcgcggggcccggggaggtggctgagctccccggggatgagagtggcaccccaggcgatgggcgaccaaatctgcgcatgaagttccagggcgccttccgcaagggggtgcccaaccccatcgatctgctggagtccaccctatatgagtcctcggtggtgcctgggcccaagaaagcacccatggactcactgtttgactacggcacctatcgtcaccactccagtgacaacaagaggtggaggaagaagatcatagagaagcagccgcagagccccaaagcccctgcccctcagccgccccccatcctcaaagtcttcaaccggcctatcctctttgacatcgtgtcccggggctccactgctgacctggacgggctgctcccattcttgctgacccacaagaaacgcctaactgatgaggagtttcgagagccatctacggggaagacctgcctgcccaaggccttgctgaacctgagcaatggccgcaacgacaccatccctgtgctgctggacatcgcggagcgcaccggcaacatgagggagttcattaactcgcccttccgtgacatctactatcgaggtcagacagccctgcacatcgccattgagcgtcgctgcaaacactacgtggaacttctcgtggcccagggagctgatgtccacgcccaggcccgtgggcgcttcttccagcccaaggatgaggggggctacttctactttggggagctgcccctgtcgctggctgcctgcaccaaccagccccacattgtcaactacctgacggagaacccccacaagaaggcggacatgcggcgccaggactcgcgaggcaacacagtgctgcatgcgctggtggccattgctgacaacacccgtgagaacaccaagtttgttaccaagatgtacgacctgctgctgctcaagtgtgcccgcctcttccccgacagcaacctggaggccgtgctcaacaacgacggcctctcgcccctcatgatggctgccaagacgggcaagattgggatctttcagcacatcatccggcgggaggtgacggatgaggacacacggcacctgtcccgcaagttcaaggactgggcctatgggccagtgtattcctcgctttatgacctctcctccctggacacgtgtggggaagaggcctccgtgctggagatcctggtgtacaacagcaagattgagaaccgccacgagatgctggctgtggagcccatcaatgaactgctgcgggacaagtggcgcaagttcggggccgtctccttctacatcaacgtggtctcctacctgtgtgccatggtcatcttcactctcaccgcctactaccagccgctggagggcacaccgccgtacccttaccgcaccacggtggactacctgcggctggctggcgaggtcattacgctcttcactggggtcctgttcttcttcaccaacatcaaagacttgttcatgaagaaatgccctggagtgaattctctcttcattgatggctccttccagctgctctacttcatctactctgtcctggtgatcgtctcagcagccctctacctggcagggatcgaggcctacctggccgtgatggtctttgccctggtcctgggctggatgaatgccctttacttcacccgtgggctgaagctgacggggacctatagcatcatgatccagaagattctcttcaaggaccttttccgattcctgctcgtctacttgctcttcatgatcggctacgcttcagccctggtctccctcctgaacccgtgtgccaacatgaaggtgtgcaatgaggaccagaccaactgcacagtgcccacttacccctcgtgccgtgacagcgagaccttcagcaccttcctcctggacctgtttaagctgaccatcggcatgggcgacctggagatgctgagcagcaccaagtaccccgtggtcttcatcatcctgctggtgacctacatcatcctcacctttgtgctgctcctcaacatgctcattgccctcatgggcgagacagtgggccaggtctccaaggagagcaagcacatctggaagctgcagtgggccaccaccatcctggacattgagcgctccttccccgtattcctgaggaaggccttccgctctggggagatggtcaccgtgggcaagagctcggacggcactcctgaccgcaggtggtgcttcagggtggatgaggtgaactggtctcactggaaccagaacttgggcatcatcaacgaggacccgggcaagaatgagacctaccagtattatggcttctcgcataccgtgggccgcctccgcagggatcgctggtcctcggtggtaccccgcgtggtggaactgaacaagaactcgaacccggacgaggtggtggtgcctctggacagcatggggaacccccgctgcgatggccaccagcagggttacccccgcaagtggaggactgatgacgccccgctctagggactgcagcccagccccagcttctctgcccactcatttctagtccagccgcatttcagcagtgccttctggggtgtccccccacaccctgctttggccccagaggcgagggaccagtggaggtgccagggaggccccaggaccctgtggtcccctggctctgcctccccaccctggggtgggggctcccggccacctgtcttgctcctatggagtcacataagccaacgccagagcccctccacctcaggccccagcccctgcctctccattatttatttgctctgctctcaggaagcgacgtgacccctgccccagctggaacctggcagaggccttaggaccccgttccaagtgcactgcccggccaagccccagcctcagcctgcgcctgagctgcatgcgccaccatttttggcagcgtggcagctttgcaaggggctggggccctcggcgtggggccatgccttctgtgtgttctgtagtgtctgggatttgccggtgctcaataaatgtttattcattgacggtggaaaaaaaaaaaa

SEQ ID NO: 5 - DNA, 3051 bp, Homo sapiens
gctgagcagtgcagacgggcctggggcaggcatggcggattccagcgaaggcccccgcgcggggcccggggaggtggctgagctccccggggatgagagtggcaccccaggtggggaggcttttcctctctcctccctggccaatctgtttgagggggaggatggctccctttcgccctcaccggctgatgccagtcgccctgctggcccaggcgatgggcgaccaaatctgcgcatgaagttccagggcgccttccgcaagggggtgcccaaccccatcgatctgctggagtccaccctatatgagtcctcggtggtgcctgggcccaagaaagcacccatggactcactgtttgactacggcacctatcgtcaccactccagtgacaacaagaggtggaggaagaagatcatagagaagcagccgcagagccccaaagcccctgcccctcagccgccccccatcctcaaagtcttcaaccggcctatcctctttgacatcgtgtcccggggctccactgctgacctggacgggctgctcccattcttgctgacccacaagaaacgcctaactgatgaggagtttcgagagccatctacggggaagacctgcctgcccaaggccttgctgaacctgagcaatggccgcaacgacaccatccctgtgctgctggacatcgcggagcgcaccggcaacatgagggagttcattaactcgcccttccgtgacatctactatcgaggggagctgcccctgtcgctggctgcctgcaccaaccagccccacattgtcaactacctgacggagaacccccacaagaaggcggacatgcggcgccaggactcgcgaggcaacacagtgctgcatgcgctggtggccattgctgacaacacccgtgagaacaccaagtttgttaccaagatgtacgacctgctgctgctcaagtgtgcccgcctcttccccgacagcaacctggaggccgtgctcaacaacgacggcctctcgcccctcatgatggctgccaagacgggcaagattgggatctttcagcacatcatccggcgggaggtgacggatgaggacacacggcacctgtcccgcaagttcaaggactgggcctatgggccagtgtattcctcgctttatgacctctcctccctggacacgtgtggggaagaggcctccgtgctggagatcctggtgtacaacagcaagattgagaaccgccacgagatgctggctgtggagcccatcaatgaactgctgcgggacaagtggcgcaagttcggggccgtctccttctacatcaacgtggtctcctacctgtgtgccatggtcatcttcactctcaccgcctactaccagccgctggagggcacaccgccgtacccttaccgcaccacggtggactacctgcggctggctggcgaggtcattacgctcttcactggggtcctgttcttcttcaccaacatcaaagacttgttcatgaagaaatgccctggagtgaattctctcttcattgatggctccttccagctgctctacttcatctactctgtcctggtgatcgtctcagcagccctctacctggcagggatcgaggcctacctggccgtgatggtctttgccctggtcctgggctggatgaatgccctttacttcacccgtgggctgaagctgacggggacctatagcatcatgatccagaagattctcttcaaggaccttttccgattcctgctcgtctacttgctcttcatgatcggctacgcttcagccctggtctccctcctgaacccgtgtgccaacatgaaggtgtgcaatgaggaccagaccaactgcacagtgcccacttacccctcgtgccgtgacagcgagaccttcagcaccttcctcctggacctgtttaagctgaccatcggcatgggcgacctggagatgctgagcagcaccaagtaccccgtggtcttcatcatcctgctggtgacctacatcatcctcacctttgtgctgctcctcaacatgctcattgccctcatgggcgagacagtgggccaggtctccaaggagagcaagcacatctggaagctgcagtgggccaccaccatcctggacattgagcgctccttccccgtattcctgaggaaggccttccgctctggggagatggtcaccgtgggcaagagctcggacggcactcctgaccgcaggtggtgcttcagggtggatgaggtgaactggtctcactggaaccagaacttgggcatcatcaacgaggacccgggcaagaatgagacctaccagtattatggcttctcgcataccgtgggccgcctccgcagggatcgctggtcctcggtggtaccccgcgtggtggaactgaacaagaactcgaacccggacgaggtggtggtgcctctggacagcatggggaacccccgctgcgatggccaccagcagggttacccccgcaagtggaggactgatgacgccccgctctagggactgcagcccagccccagcttctctgcccactcatttctagtccagccgcatttcagcagtgccttctggggtgtccccccacaccctgctttggccccagaggcgagggaccagtggaggtgccagggaggccccaggaccctgtggtcccctggctctgcctccccaccctggggtgggggctcccggccacctgtcttgctcctatggagtcacataagccaacgccagagcccctccacctcaggccccagcccctgcctctccattatttatttgctctgctctcaggaagcgacgtgacccctgccccagctggaacctggcagaggccttaggaccccgttccaagtgcactgcccggccaagccccagcctcagcctgcgcctgagctgcatgcgccaccatttttggcagcgtggcagctttgcaaggggctggggccctcggcgtggggccatgccttctgtgtgttctgtagtgtctgggatttgccggtgctcaataaatgtttattcattgacggtggaaaaaaaaaaaa

SEQ ID NO: 6 - DNA, 23 bp, Artificial Sequence
  antisense oligonucleotide
catcaccaggatctgccatactg

SEQ ID NO: 7 - DNA, 21 bp, Artificial Sequence
  siRNA
ucuaccaguacuauggcuutt

SEQ ID NO: 8 - DNA, 21 bp, Artificial Sequence
  siRNA
ttagauggucaugauaccgaa